European Patent Specification EP 3 040 417 B1, published December 13, 2023. Title: Macrocyclic Peptide, Method of Producing the Same, and Screening method using Macrocyclic Peptide Library. Applicant: The University of Tokyo. The sequence listing filed with the application follows.

SEQUENCE LISTING (64 sequences)

SEQ ID NO: 1 - RNA, 24 nt, Artificial
  Synthesized RNA.
  misc_feature (4)..(5): "n" stands for a, u, g or c.
  misc_feature (4)..(6): "nnu" is repeated 2 to 3 times.
  misc_feature (10)..(11): "n" stands for a, u, g or c.
  misc_feature (10)..(12): "nnu" is repeated 5 to 7 times.
  misc_feature (16)..(17): "n" stands for a, u, g or c.
  misc_feature (16)..(18): "nnu" is repeated 2 to 3 times.
augnnuaugnnuaugnnuuguggc

SEQ ID NO: 2 - RNA, 21 nt, Artificial
  Synthesized RNA.
  misc_feature (4)..(5): "n" stands for a, u, g or c.
  misc_feature (4)..(6): "nnu" is repeated 2 to 4 times.
  misc_feature (10)..(11): "n" stands for a, u, g or c.
  misc_feature (10)..(12): "nnu" is repeated 5 to 7 times.
augnnnaugnnnauguguggc

SEQ ID NO: 3 - protein, 14 aa, Artificial
  Synthesized peptide.
  MOD_RES (1)..(1): Chloroacetyl-D-phenylalanine.
  misc_feature (4)..(4): "Xaa" stands for 2-Aminoheptonic acid.
  misc_feature (11)..(11): "Xaa" stands for 2-Aminoheptonic acid.
FNAXYPYRPPXTSC

SEQ ID NO: 4 - protein, 14 aa, Artificial
  Synthesized peptide.
  MOD_RES (1)..(1): Chloroacetyl-D-phenylalanine.
  MISC_FEATURE (4)..(4): "Xaa" stands for 2-Aminoheptonic acid.
  MISC_FEATURE (11)..(11): "Xaa" stands for 2-Aminoheptonic acid.
FDAXYPFRPPXAHC

SEQ ID NO: 5 - protein, 15 aa, Artificial
  Synthesized peptide.
  MOD_RES (1)..(1): Chloroacetyl-D-phenylalanine.
  MISC_FEATURE (5)..(5): "Xaa" stands for 2-Aminoheptonic acid.
  MISC_FEATURE (11)..(11): "Xaa" stands for 2-Aminoheptonic acid.
FYRCXHPVPVXPTPC

SEQ ID NO: 6 - protein, 14 aa, Artificial
  Synthesized peptide.
  MOD_RES (1)..(1): Chloroacetyl-D-phenylalanine.
  MISC_FEATURE (4)..(4): "Xaa" stands for 2-Aminoheptonic acid.
  MISC_FEATURE (11)..(11): "Xaa" stands for 2-Aminoheptonic acid.
FNAXYPFRPPXTTC

SEQ ID NO: 7 - protein, 15 aa, Artificial
  Synthesized peptide.
  MOD_RES (1)..(1): Chloroacetyl-D-phenylalanine.
  MISC_FEATURE (5)..(5): "Xaa" stands for 2-Aminoheptonic acid.
  MISC_FEATURE (11)..(11): "Xaa" stands for 2-Aminoheptonic acid.
FYRCXYPVPRXTRPC

SEQ ID NO: 8 - protein, 17 aa, Artificial
  Synthesized peptide.
  MOD_RES (1)..(1): Chloroacetyl-D-phenylalanine.
  MISC_FEATURE (5)..(5): "Xaa" stands for 2-Aminoheptonic acid.
  MISC_FEATURE (13)..(13): "Xaa" stands for 2-Aminoheptonic acid.
FYRCXYPLPSPPXTPHC

SEQ ID NO: 9 - protein, 14 aa, Artificial
  Synthesized peptide.
  MOD_RES (1)..(1): Chloroacetyl-D-phenylalanine.
  MISC_FEATURE (5)..(5): "Xaa" stands for 2-Aminoheptonic acid.
  MISC_FEATURE (13)..(13): "Xaa" stands for 2-Aminoheptonic acid.
FYRCXYPIPRPPXC

SEQ ID NO: 10 - protein, 14 aa, Artificial
  Synthesized peptide.
  MOD_RES (1)..(1): Chloroacetyl-D-phenylalanine.
  MISC_FEATURE (5)..(5): "Xaa" stands for 2-Aminoheptonic acid.
  MISC_FEATURE (13)..(13): "Xaa" stands for 2-Aminoheptonic acid.
FYRCXNPIPALPXC

SEQ ID NO: 11 - protein, 14 aa, Artificial
  Synthesized peptide.
  MOD_RES (1)..(1): Chloroacetyl-D-phenylalanine.
  MISC_FEATURE (5)..(5): "Xaa" stands for 2-Aminoheptonic acid.
  MISC_FEATURE (13)..(13): "Xaa" stands for 2-Aminoheptonic acid.
FYRCXHPVPRPPXC

SEQ ID NO: 12 - protein, 15 aa, Artificial
  Synthesized peptide.
  MOD_RES (1)..(1): Chloroacetyl-D-phenylalanine.
  MISC_FEATURE (6)..(6): "Xaa" stands for 2-Aminoheptonic acid.
  MISC_FEATURE (14)..(14): "Xaa" stands for 2-Aminoheptonic acid.
FVSRSXFDALPNNXC

SEQ ID NO: 13 - protein, 15 aa, Artificial
  Synthesized peptide.
  MOD_RES (1)..(1): Chloroacetyl-D-phenylalanine.
  MISC_FEATURE (6)..(6): "Xaa" stands for 2-Aminoheptonic acid.
  MISC_FEATURE (14)..(14): "Xaa" stands for 2-Aminoheptonic acid.
FPSIRXAFPHTNPXC

SEQ ID NO: 14 - DNA, 49 bp, Artificial
  Synthesized primer.
gtaatacgactcactataggcggggtggagcagcctggtagctcgtcgg

SEQ ID NO: 15 - DNA, 44 bp, Artificial
  Synthesized primer.
gaaccgacgatcttcgggttatgagcccgacgagctaccagcct

SEQ ID NO: 16 - DNA, 22 bp, Artificial
  Synthesized primer.
ggcgtaatacgactcactatag

SEQ ID NO: 17 - DNA, 38 bp, Artificial
  Synthesized primer.
tggttgcgggggccggatttgaaccgacgatcttcggg

SEQ ID NO: 18 - DNA, 20 bp, Artificial
  Synthesized primer.
tggttgcgggggcccgattt

SEQ ID NO: 19 - DNA, 49 bp, Artificial
  Synthesized primer.
gtaatacgactcactataggctctgtagttcagtcggtagaacggcgga

SEQ ID NO: 20 - DNA, 43 bp, Artificial
  Synthesized primer.
gaaccagtgacatacggattatgagtccgccgttctaccgact

SEQ ID NO: 21 - DNA, 38 bp, Artificial
  Synthesized primer.
tggcggctctgactggactcgaaccagtgacatacgga

SEQ ID NO: 22 - DNA, 20 bp, Artificial
  Synthesized primer.
tggcggctctgactggactc

SEQ ID NO: 23 - DNA, 36 bp, Artificial
  Synthesized primer.
gtaatacgactcactataggatcgaaagatttccgc

SEQ ID NO: 24 - DNA, 45 bp, Artificial
  Synthesized primer.
acctaacgctaatcccctttcggggccgcggaaatctttcgatcc

SEQ ID NO: 25 - DNA, 18 bp, Artificial
  Synthesized primer.
acctaacgctaatcccct

SEQ ID NO: 26 - DNA, 43 bp, Artificial
  Synthesized primer.
  misc_feature (21)..(21): "n" stands for uracil.
gaaccagtgacatacggattnggagtccgccgttctaccgact

SEQ ID NO: 27 - DNA, 46 bp, Artificial
  Synthesized primer.
taatacgactcactatagggttaactttaacaaggagaaaaacatg

SEQ ID NO: 28 - DNA, 47 bp, Artificial
  Synthesized primer.
aatcggcggaatagacttggtcatcatgtttttctccttgttaaagt

SEQ ID NO: 29 - DNA, 22 bp, Artificial
  Synthesized primer.
ggcgtaatacgactcactatag

SEQ ID NO: 30 - DNA, 49 bp, Artificial
  Synthesized primer.
cgtcgtccttgtagtcacagtccggaaacataatcggcggaatagactt

SEQ ID NO: 31 - DNA, 29 bp, Artificial
  Synthesized primer.
ttacttgtcgtcgtcgtccttgtagtcac

SEQ ID NO: 32 - DNA, 49 bp, Artificial
  Synthesized primer.
taatacgactcactatagggttgaactttaagtaggagatatatccatg

SEQ ID NO: 33 - DNA, 39 bp, Artificial
  Synthesized primer.
tttccgccccccgtcctaagacccagacccagacccaca

SEQ ID NO: 34 - DNA, 78 bp, Artificial
  Synthesized primer.
  misc_feature (23)..(24): "n" stands for a, c, g or t.
  misc_feature (26)..(27): "n" stands for a, c, g or t.
  misc_feature (32)..(33): "n" stands for a, c, g or t.
  misc_feature (35)..(36): "n" stands for a, c, g or t.
  misc_feature (38)..(39): "n" stands for a, c, g or t.
  misc_feature (41)..(42): "n" stands for a, c, g or t.
  misc_feature (44)..(45): "n" stands for a, c, g or t.
  misc_feature (50)..(51): "n" stands for a, c, g or t.
  misc_feature (53)..(54): "n" stands for a, c, g or t.
agacccagacccagacccacaannanncatannannannannanncatannanncatggatatatctcctacttaaag

SEQ ID NO: 35 - DNA, 81 bp, Artificial
  Synthesized primer.
  misc_feature (23)..(24): "n" stands for a, c, g or t.
  misc_feature (26)..(27): "n" stands for a, c, g or t.
  misc_feature (32)..(33): "n" stands for a, c, g or t.
  misc_feature (35)..(36): "n" stands for a, c, g or t.
  misc_feature (38)..(39): "n" stands for a, c, g or t.
  misc_feature (41)..(42): "n" stands for a, c, g or t.
  misc_feature (44)..(45): "n" stands for a, c, g or t.
  misc_feature (47)..(48): "n" stands for a, c, g or t.
  misc_feature (53)..(54): "n" stands for a, c, g or t.
  misc_feature (56)..(57): "n" stands for a, c, g or t.
agacccagacccagacccacaannanncatannannannannannanncatannanncatggatatatctcctacttaaag

SEQ ID NO: 36 - DNA, 83 bp, Artificial
  Synthesized primer.
  misc_feature (23)..(24): "n" stands for a, c, g or t.
  misc_feature (26)..(27): "n" stands for a, c, g or t.
  misc_feature (32)..(33): "n" stands for a, c, g or t.
  misc_feature (35)..(36): "n" stands for a, c, g or t.
  misc_feature (38)..(39): "n" stands for a, c, g or t.
  misc_feature (41)..(44): "n" stands for a, c, g or t.
  misc_feature (46)..(47): "n" stands for a, c, g or t.
  misc_feature (49)..(50): "n" stands for a, c, g or t.
  misc_feature (55)..(56): "n" stands for a, c, g or t.
  misc_feature (58)..(59): "n" stands for a, c, g or t.
agacccagacccagacccacaannanncatannannannannnnannanncatannanncatggatatatctcctacttaaag

SEQ ID NO: 37 - DNA, 81 bp, Artificial
  Synthesized primer.
  misc_feature (23)..(24): "n" stands for a, c, g or t.
  misc_feature (26)..(27): "n" stands for a, c, g or t.
  misc_feature (29)..(30): "n" stands for a, c, g or t.
  misc_feature (35)..(36): "n" stands for a, c, g or t.
  misc_feature (38)..(39): "n" stands for a, c, g or t.
  misc_feature (41)..(42): "n" stands for a, c, g or t.
  misc_feature (44)..(45): "n" stands for a, c, g or t.
  misc_feature (47)..(48): "n" stands for a, c, g or t.
  misc_feature (53)..(54): "n" stands for a, c, g or t.
  misc_feature (56)..(57): "n" stands for a, c, g or t.
agacccagacccagacccacaannannanncatannannannannanncatannanncatggatatatctcctacttaaag

SEQ ID NO: 38 - DNA, 84 bp, Artificial
  Synthesized primer.
  misc_feature (23)..(24): "n" stands for a, c, g or t.
  misc_feature (26)..(27): "n" stands for a, c, g or t.
  misc_feature (29)..(30): "n" stands for a, c, g or t.
  misc_feature (35)..(36): "n" stands for a, c, g or t.
  misc_feature (38)..(39): "n" stands for a, c, g or t.
  misc_feature (41)..(42): "n" stands for a, c, g or t.
  misc_feature (44)..(45): "n" stands for a, c, g or t.
  misc_feature (47)..(48): "n" stands for a, c, g or t.
  misc_feature (50)..(51): "n" stands for a, c, g or t.
  misc_feature (56)..(57): "n" stands for a, c, g or t.
  misc_feature (59)..(60): "n" stands for a, c, g or t.
agacccagacccagacccacaannannanncatannannannannannanncatannanncatggatatatctcctacttaaag

SEQ ID NO: 39 - DNA, 86 bp, Artificial
  Synthesized primer.
  misc_feature (23)..(24): "n" stands for a, c, g or t.
  misc_feature (26)..(27): "n" stands for a, c, g or t.
  misc_feature (29)..(30): "n" stands for a, c, g or t.
  misc_feature (35)..(36): "n" stands for a, c, g or t.
  misc_feature (38)..(39): "n" stands for a, c, g or t.
  misc_feature (41)..(42): "n" stands for a, c, g or t.
  misc_feature (44)..(45): "n" stands for a, c, g or t.
  misc_feature (47)..(48): "n" stands for a, c, g or t.
  misc_feature (50)..(51): "n" stands for a, c, g or t.
  misc_feature (53)..(54): "n" stands for a, c, g or t.
  misc_feature (59)..(60): "n" stands for a, c, g or t.
  misc_feature (62)..(63): "n" stands for a, c, g or t.
agacccagacccagacccacaannannanncatannannannannannannanncatannanncatggatatatctcctacttaaa

SEQ ID NO: 40 - DNA, 84 bp, Artificial
  Synthesized primer.
  misc_feature (23)..(24): "n" stands for a, c, g or t.
  misc_feature (26)..(27): "n" stands for a, c, g or t.
  misc_feature (29)..(30): "n" stands for a, c, g or t.
  misc_feature (35)..(36): "n" stands for a, c, g or t.
  misc_feature (38)..(39): "n" stands for a, c, g or t.
  misc_feature (41)..(42): "n" stands for a, c, g or t.
  misc_feature (44)..(45): "n" stands for a, c, g or t.
  misc_feature (47)..(48): "n" stands for a, c, g or t.
  misc_feature (53)..(54): "n" stands for a, c, g or t.
  misc_feature (56)..(57): "n" stands for a, c, g or t.
  misc_feature (59)..(60): "n" stands for a, c, g or t.
agacccagacccagacccacaannannanncatannannannannanncatannannanncatggatatatctcctacttaaag

SEQ ID NO: 41 - DNA, 87 bp, Artificial
  Synthesized primer.
  misc_feature (23)..(24): "n" stands for a, c, g or t.
  misc_feature (26)..(27): "n" stands for a, c, g or t.
  misc_feature (29)..(30): "n" stands for a, c, g or t.
  misc_feature (35)..(36): "n" stands for a, c, g or t.
  misc_feature (38)..(39): "n" stands for a, c, g or t.
  misc_feature (41)..(42): "n" stands for a, c, g or t.
  misc_feature (44)..(45): "n" stands for a, c, g or t.
  misc_feature (47)..(48): "n" stands for a, c, g or t.
  misc_feature (50)..(51): "n" stands for a, c, g or t.
  misc_feature (56)..(57): "n" stands for a, c, g or t.
  misc_feature (59)..(60): "n" stands for a, c, g or t.
  misc_feature (62)..(63): "n" stands for a, c, g or t.
agacccagacccagacccacaannannanncatannannannannannanncatannannanncatggatatatctcctacttaaag

SEQ ID NO: 42 - DNA, 89 bp, Artificial
  Synthesized primer.
  misc_feature (23)..(24): "n" stands for a, c, g or t.
  misc_feature (26)..(27): "n" stands for a, c, g or t.
  misc_feature (29)..(30): "n" stands for a, c, g or t.
  misc_feature (35)..(36): "n" stands for a, c, g or t.
  misc_feature (38)..(39): "n" stands for a, c, g or t.
  misc_feature (41)..(42): "n" stands for a, c, g or t.
  misc_feature (44)..(45): "n" stands for a, c, g or t.
  misc_feature (47)..(48): "n" stands for a, c, g or t.
  misc_feature (50)..(51): "n" stands for a, c, g or t.
  misc_feature (53)..(54): "n" stands for a, c, g or t.
  misc_feature (59)..(60): "n" stands for a, c, g or t.
  misc_feature (62)..(63): "n" stands for a, c, g or t.
  misc_feature (65)..(66): "n" stands for a, c, g or t.
agacccagacccagacccacaannannanncatannannannannannannanncatannannanncatggatatatctcctacttaag

SEQ ID NO: 43 - DNA, 72 bp, Artificial
  Synthesized primer.
  misc_feature (26)..(27): "n" stands for a, c, g or t.
  misc_feature (29)..(30): "n" stands for a, c, g or t.
  misc_feature (32)..(33): "n" stands for a, c, g or t.
  misc_feature (35)..(36): "n" stands for a, c, g or t.
  misc_feature (38)..(39): "n" stands for a, c, g or t.
  misc_feature (44)..(45): "n" stands for a, c, g or t.
  misc_feature (47)..(48): "n" stands for a, c, g or t.
agacccagacccagacccacacatannannannannanncatannanncatggatatatctcctacttaaag

SEQ ID NO: 44 - DNA, 75 bp, Artificial
  Synthesized primer.
  misc_feature (26)..(27): "n" stands for a, c, g or t.
  misc_feature (29)..(30): "n" stands for a, c, g or t.
  misc_feature (32)..(33): "n" stands for a, c, g or t.
  misc_feature (35)..(36): "n" stands for a, c, g or t.
  misc_feature (38)..(39): "n" stands for a, c, g or t.
  misc_feature (41)..(42): "n" stands for a, c, g or t.
  misc_feature (47)..(48): "n" stands for a, c, g or t.
  misc_feature (50)..(51): "n" stands for a, c, g or t.
agacccagacccagacccacacatannannannannannanncatannanncatggatatatctcctacttaaag

SEQ ID NO: 45 - DNA, 78 bp, Artificial
  Synthesized primer.
  misc_feature (26)..(27): "n" stands for a, c, g or t.
  misc_feature (29)..(30): "n" stands for a, c, g or t.
  misc_feature (32)..(33): "n" stands for a, c, g or t.
  misc_feature (35)..(36): "n" stands for a, c, g or t.
  misc_feature (38)..(39): "n" stands for a, c, g or t.
  misc_feature (41)..(42): "n" stands for a, c, g or t.
  misc_feature (44)..(45): "n" stands for a, c, g or t.
  misc_feature (50)..(51): "n" stands for a, c, g or t.
  misc_feature (53)..(54): "n" stands for a, c, g or t.
agacccagacccagacccacacatannannannannannannanncatannanncatggatatatctcctacttaaag

SEQ ID NO: 46 - DNA, 75 bp, Artificial
  Synthesized primer.
  misc_feature (26)..(27): "n" stands for a, c, g or t.
  misc_feature (29)..(30): "n" stands for a, c, g or t.
  misc_feature (32)..(33): "n" stands for a, c, g or t.
  misc_feature (35)..(36): "n" stands for a, c, g or t.
  misc_feature (38)..(39): "n" stands for a, c, g or t.
  misc_feature (44)..(45): "n" stands for a, c, g or t.
  misc_feature (47)..(48): "n" stands for a, c, g or t.
  misc_feature (50)..(51): "n" stands for a, c, g or t.
agacccagacccagacccacacatannannannannanncatannannanncatggatatatctcctacttaaag

SEQ ID NO: 47 - DNA, 78 bp, Artificial
  Synthesized primer.
  misc_feature (26)..(27): "n" stands for a, c, g or t.
  misc_feature (29)..(30): "n" stands for a, c, g or t.
  misc_feature (32)..(33): "n" stands for a, c, g or t.
  misc_feature (35)..(36): "n" stands for a, c, g or t.
  misc_feature (38)..(39): "n" stands for a, c, g or t.
  misc_feature (41)..(42): "n" stands for a, c, g or t.
  misc_feature (47)..(48): "n" stands for a, c, g or t.
  misc_feature (50)..(51): "n" stands for a, c, g or t.
  misc_feature (53)..(54): "n" stands for a, c, g or t.
agacccagacccagacccacacatannannannannannanncatannannanncatggatatatctcctacttaaag

SEQ ID NO: 48 - DNA, 81 bp, Artificial
  Synthesized primer.
  misc_feature (26)..(27): "n" stands for a, c, g or t.
  misc_feature (29)..(30): "n" stands for a, c, g or t.
  misc_feature (32)..(33): "n" stands for a, c, g or t.
  misc_feature (35)..(36): "n" stands for a, c, g or t.
  misc_feature (38)..(39): "n" stands for a, c, g or t.
  misc_feature (41)..(42): "n" stands for a, c, g or t.
  misc_feature (44)..(45): "n" stands for a, c, g or t.
  misc_feature (50)..(51): "n" stands for a, c, g or t.
  misc_feature (53)..(54): "n" stands for a, c, g or t.
  misc_feature (56)..(57): "n" stands for a, c, g or t.
agacccagacccagacccacacatannannannannannannanncatannannanncatggatatatctcctacttaaag

SEQ ID NO: 49 - DNA, 78 bp, Artificial
  Synthesized primer.
  misc_feature (26)..(27): "n" stands for a, c, g or t.
  misc_feature (29)..(30): "n" stands for a, c, g or t.
  misc_feature (32)..(33): "n" stands for a, c, g or t.
  misc_feature (35)..(36): "n" stands for a, c, g or t.
  misc_feature (38)..(39): "n" stands for a, c, g or t.
  misc_feature (44)..(45): "n" stands for a, c, g or t.
  misc_feature (47)..(48): "n" stands for a, c, g or t.
  misc_feature (50)..(51): "n" stands for a, c, g or t.
  misc_feature (53)..(54): "n" stands for a, c, g or t.
agacccagacccagacccacacatannannannannanncatannannannanncatggatatatctcctacttaaag

SEQ ID NO: 50 - DNA, 81 bp, Artificial
  Synthesized primer.
  misc_feature (26)..(27): "n" stands for a, c, g or t.
  misc_feature (29)..(30): "n" stands for a, c, g or t.
  misc_feature (32)..(33): "n" stands for a, c, g or t.
  misc_feature (35)..(36): "n" stands for a, c, g or t.
  misc_feature (38)..(39): "n" stands for a, c, g or t.
  misc_feature (41)..(42): "n" stands for a, c, g or t.
  misc_feature (47)..(48): "n" stands for a, c, g or t.
  misc_feature (50)..(51): "n" stands for a, c, g or t.
  misc_feature (53)..(54): "n" stands for a, c, g or t.
  misc_feature (56)..(57): "n" stands for a, c, g or t.
agacccagacccagacccacacatannannannannannanncatannannannanncatggatatatctcctacttaaag

SEQ ID NO: 51 - DNA, 84 bp, Artificial
  Synthesized primer.
  misc_feature (26)..(27): "n" stands for a, c, g or t.
  misc_feature (29)..(30): "n" stands for a, c, g or t.
  misc_feature (32)..(33): "n" stands for a, c, g or t.
  misc_feature (35)..(36): "n" stands for a, c, g or t.
  misc_feature (38)..(39): "n" stands for a, c, g or t.
  misc_feature (41)..(42): "n" stands for a, c, g or t.
  misc_feature (44)..(45): "n" stands for a, c, g or t.
  misc_feature (50)..(51): "n" stands for a, c, g or t.
  misc_feature (53)..(54): "n" stands for a, c, g or t.
  misc_feature (56)..(57): "n" stands for a, c, g or t.
  misc_feature (59)..(60): "n" stands for a, c, g or t.
agacccagacccagacccacacatannannannannannannanncatannannannanncatggatatatctcctacttaaag

SEQ ID NO: 52 - DNA, 49 bp, Artificial; identical to SEQ ID NO: 32
  Synthesized primer.

SEQ ID NO: 53 - DNA, 39 bp, Artificial; identical to SEQ ID NO: 33
  Synthesized primer.

SEQ ID NO: 54 - RNA, 69 nt, Artificial
  Synthesized DNA.
auguggaccaagucuauuccgccgauuugguuuccggacugugacuacaaggacgacgacgacaaguaa

SEQ ID NO: 55 - protein, 22 aa, Artificial
  Synthesized peptide.
  MOD_RES (1)..(1): Chloroacetyl-D-phenylalanine.
  MISC_FEATURE (2)..(2): "Xaa" stands for 2-Aminoheptonic acid.
  MISC_FEATURE (10)..(10): "Xaa" stands for 2-Aminoheptonic acid.
FXTKSIPPIXFPDCDYKDDDDK

SEQ ID NO: 56 - protein, 22 aa, Artificial
  Synthesized peptide.
  MISC_FEATURE (1)..(1): Chloroacetyl-D-phenylalanine.
FSTKSIPPISFPDCDYKDDDDK

SEQ ID NO: 57 - RNA, 18 nt, Artificial
  Synthesized RNA.
uaauacgacucacuauag

SEQ ID NO: 58 - RNA, 10 nt, Artificial
  Synthesized RNA.
uuaacuuuaa

SEQ ID NO: 59 - RNA, 7 nt, Artificial
  Synthesized RNA.
aaggaga

SEQ ID NO: 60 - RNA, 18 nt, Artificial
  Synthesized RNA.
ggcagcggcagcggcagc

SEQ ID NO: 61 - RNA, 18 nt, Artificial
  Synthesized RNA.
uaggacggggggcggaaa

SEQ ID NO: 62 - DNA, 49 bp, Artificial; identical to SEQ ID NO: 32
  Synthesized primer.

SEQ ID NO: 63 - DNA, 39 bp, Artificial; identical to SEQ ID NO: 33
  Synthesized primer.

SEQ ID NO: 64 - DNA, 16 bp, Artificial
  Synthesized DNA.
ctcccgccccccgtcc